European Patent Specification EP 3 564 361 B1, published December 25, 2024. Title: Liver organoid, uses thereof and culture method for obtaining them. Applicant: Koninklijke Nederlandse Akademie van Wetenschappen. Application PCT/IB2011/002167. The sequence listing filed with the application follows.

SEQUENCE LISTING (26 sequences)

SEQ ID NO: 1 - DNA, 23 bp, Artificial Sequence
  Primer
tggtcaaacgcctctccttgctg

SEQ ID NO: 2 - DNA, 20 bp, Artificial Sequence
  primer
actgggccaaaatcccgccg

SEQ ID NO: 3 - DNA, 19 bp, Artificial Sequence
  primer
gaattaccaagactccagg

SEQ ID NO: 4 - DNA, 20 bp, Artificial Sequence
  primer
tgagacaatacttccggagg

SEQ ID NO: 5 - DNA, 20 bp, Artificial Sequence
  primer
gtcctacagattgacaatgc

SEQ ID NO: 6 - DNA, 20 bp, Artificial Sequence
  primer
cacgctctggatctgtgaca

SEQ ID NO: 7 - DNA, 20 bp, Artificial Sequence
  primer
gcgcagatgacagggcggaa

SEQ ID NO: 8 - DNA, 20 bp, Artificial Sequence
  primer
gtgccgtagcatgcgggagg

SEQ ID NO: 9 - DNA, 20 bp, Artificial Sequence
  primer
agcgatcacgcaacgtggca

SEQ ID NO: 10 - DNA, 24 bp, Artificial Sequence
  primer
ggcttcgctgggacacagatcttt

SEQ ID NO: 11 - DNA, 18 bp, Artificial Sequence
  primer
ttcaacagatgcattacc

SEQ ID NO: 12 - DNA, 18 bp, Artificial Sequence
  primer
tctttgcccgcgatgatg

SEQ ID NO: 13 - DNA, 20 bp, Artificial Sequence
  primer
acgactggagcgcacgagac

SEQ ID NO: 14 - DNA, 20 bp, Artificial Sequence
  primer
agggctggctgtggcagaga

SEQ ID NO: 15 - DNA, 21 bp, Artificial Sequence
  primer
tttggcagtggctgaaaggca

SEQ ID NO: 16 - DNA, 20 bp, Artificial Sequence
  primer
gggcccaggatccgctgact

SEQ ID NO: 17 - DNA, 21 bp, Artificial Sequence
  primer
actccccgtagaaggcagcga

SEQ ID NO: 18 - DNA, 22 bp, Artificial Sequence
  primer
tctttccagccatgcctccact

SEQ ID NO: 19 - DNA, 22 bp, Artificial Sequence
  primer
ggaaatgctttgacacacattc

SEQ ID NO: 20 - DNA, 23 bp, Artificial Sequence
  primer
ggaagtcatcaaggttattataa

SEQ ID NO: 21 - DNA, 20 bp, Artificial Sequence
  primer
atggtcaaagtcctggatgc

SEQ ID NO: 22 - DNA, 20 bp, Artificial Sequence
  primer
aattcatggaacggggaaat

SEQ ID NO: 23 - DNA, 18 bp, Artificial Sequence
  primer
aagatcattggcggaaag

SEQ ID NO: 24 - DNA, 19 bp, Artificial Sequence
  primer
gagtgctcaggatgttaag

SEQ ID NO: 25 - DNA, 20 bp, Artificial Sequence
  primer
aagcttgctggtgaaaagga

SEQ ID NO: 26 - DNA, 20 bp, Artificial Sequence
  primer
ttgcgctcatcttaggcttt